European Patent Specification EP 3 865 571 B1, published December 25, 2024. Title: Mesenchymal stem cells derived from synovium and uses thereof. Applicant: Ewha University - Industry Collaboration Foundation inje university industry-academic cooperation foundation. The sequence listing filed with the application follows.

SEQUENCE LISTING (8 sequences)

SEQ ID NO: 1 - DNA, 21 bp, Artificial Sequence
  primer
cccgatctgaagaaggagagc

SEQ ID NO: 2 - DNA, 21 bp, Artificial Sequence
  primer
gttcttcaccgacttcctccg

SEQ ID NO: 3 - DNA, 23 bp, Artificial Sequence
  primer
tgaggagggctggaacaagtacc

SEQ ID NO: 4 - DNA, 23 bp, Artificial Sequence
  primer
ggaggtggtaattgcagggaaca

SEQ ID NO: 5 - DNA, 22 bp, Artificial Sequence
  primer
ttcagctatggagatgacaatc

SEQ ID NO: 6 - DNA, 20 bp, Artificial Sequence
  primer
agagtcctagagtgactgag

SEQ ID NO: 7 - DNA, 20 bp, Artificial Sequence
  primer
attgttgccatcaatgaccc

SEQ ID NO: 8 - DNA, 21 bp, Artificial Sequence
  primer
agtagaggcagggatgatgtt